European Patent Application EP 4 548 936 A1, published May 7, 2025. Title: ANTIBODY-DRUG CONJUGATES HAVING A TAILOR-MADE DRUG-TO-ANTIBODY RATIO. Applicant: BioNTech SE. The sequence listing filed with the application follows.

SEQUENCE LISTING (118 sequences)

SEQ ID NO: 1 - protein, 15 aa, synthetic construct
EPKSCDKTHTCPPCP

SEQ ID NO: 2 - protein, 12 aa, synthetic construct
ERKCCVECPPCP

SEQ ID NO: 3 - protein, 62 aa, synthetic construct
ELKTPLGDTTHTCPRCPEPKSCDTPPPCPRCPEPKSCDTPPPCPRCPEPKSCDTPPPCPRCP

SEQ ID NO: 4 - protein, 32 aa, synthetic construct
ELKTPLGDTTHTCPRCPEPKSCDTPPPCPRCP

SEQ ID NO: 5 - protein, 12 aa, synthetic construct
ESKYGPPCPSCP

SEQ ID NO: 6 - protein, 17 aa, synthetic construct
ELKTPLGDTTHTCPRCP

SEQ ID NO: 7 - protein, 15 aa, synthetic construct
EPKSCDTPPPCPRCP

SEQ ID NO: 8 - protein, 10 aa, synthetic construct
  SITE 6: note = X at position 6 can be any amino acid except C
DKTHTXPPCP

SEQ ID NO: 9 - protein, 10 aa, synthetic construct
  SITE 9: note = X at position 9 can be any amino acid except C
DKTHTCPPXP

SEQ ID NO: 10 - protein, 15 aa, synthetic construct
  SITE 5: note = X at position 5 is either C if a (human) IgG1 Fab is fused N-terminally or any amino acid except C, if any other (or no) binding domain is fused N-terminally
  SITE 11: note = X at position 11 can be any amino acid except C
EPKSXDKTHTXPPCP

SEQ ID NO: 11 - protein, 15 aa, synthetic construct
  SITE 5: note = X at position 5 is either C if a (human) IgG1 Fab is fused N-terminally or any amino acid except C, if any other (or no) binding domain is fused N-terminally
  SITE 14: note = X at position 14 can be any amino acid except C
EPKSXDKTHTCPPXP

SEQ ID NO: 12 - protein, 10 aa, synthetic construct
DKTHTCPPCP

SEQ ID NO: 13 - protein, 15 aa, synthetic construct
  SITE 5: note = X at position 5 is either C if a (human) IgG1 Fab is fused N-terminally or any amino acid except C, if any other (or no) binding domain is fused N-terminally
EPKSXDKTHTCPPCP

SEQ ID NO: 14 - protein, 12 aa, synthetic construct
  SITE 4: note = X at position 4 can be any amino acid except C
  SITE 5: note = X at position 5 can be any amino acid except C
  SITE 8: note = X at position 8 can be any amino acid except C
ERKXXVEXPPCP

SEQ ID NO: 15 - protein, 12 aa, synthetic construct
  SITE 4: note = X at position 4 can be any amino acid except C
  SITE 5: note = X at position 5 can be any amino acid except C
  SITE 11: note = X at position 11 can be any amino acid except C
ERKXXVECPPXP

SEQ ID NO: 16 - protein, 12 aa, synthetic construct
  SITE 4: note = X at position 4 can be any amino acid except C
  SITE 8: note = X at position 8 can be any amino acid except C
  SITE 11: note = X at position 11 can be any amino acid except C
ERKXCVEXPPXP

SEQ ID NO: 17 - protein, 12 aa, synthetic construct
  SITE 5: note = X at position 5 can be any amino acid except C
  SITE 11: note = X at position 11 can be any amino acid except C
  SITE 8: note = X at position 8 can be any amino acid except C
ERKCXVEXPPXP

SEQ ID NO: 18 - protein, 12 aa, synthetic construct
  SITE 4: note = X at position 4 can be any amino acid except C
  SITE 5: note = X at position 5 can be any amino acid except C
ERKXXVECPPCP

SEQ ID NO: 19 - protein, 12 aa, synthetic construct
  SITE 4: note = X at position 4 can be any amino acid except C
  SITE 8: note = X at position 8 can be any amino acid except C
ERKXCVEXPPCP

SEQ ID NO: 20 - protein, 12 aa, synthetic construct
  SITE 4: note = X at position 4 can be any amino acid except C
  SITE 11: note = X at position 11 can be any amino acid except C
ERKXCVECPPXP

SEQ ID NO: 21 - protein, 12 aa, synthetic construct
  SITE 5: note = X at position 5 can be any amino acid except C
  SITE 8: note = X at position 8 can be any amino acid except C
ERKCXVEXPPCP

SEQ ID NO: 22 - protein, 12 aa, synthetic construct
  SITE 5: note = X at position 5 can be any amino acid except C
  SITE 11: note = X at position 11 can be any amino acid except C
ERKCXVECPPXP

SEQ ID NO: 23 - protein, 12 aa, synthetic construct
  SITE 8: note = X at position 8 can be any amino acid except C
  SITE 11: note = X at position 11 can be any amino acid except C
ERKCCVEXPPXP

SEQ ID NO: 24 - protein, 12 aa, synthetic construct
  SITE 4: note = X at position 4 can be any amino acid except C
ERKXCVECPPCP

SEQ ID NO: 25 - protein, 12 aa, synthetic construct
  SITE 5: note = X at position 5 can be any amino acid except C
ERKCXVECPPCP

SEQ ID NO: 26 - protein, 12 aa, synthetic construct
  SITE 8: note = X at position 8 can be any amino acid except C
ERKCCVEXPPCP

SEQ ID NO: 27 - protein, 12 aa, synthetic construct
  SITE 11: note = X at position 11 can be any amino acid except C
ERKCCVECPPXP

SEQ ID NO: 28 - protein, 15 aa, synthetic construct
  SITE 5: note = X at position 5 can be any amino acid except C
  SITE 11: note = X at position 11 can be any amino acid except C
  VARIANT 1..11: note = any one or more of amino acids at any of positions 1-11 may be deleted
EPKSXDTPPPXPRCP

SEQ ID NO: 29 - protein, 4 aa, synthetic construct
PRCP

SEQ ID NO: 30 - protein, 15 aa, synthetic construct
  SITE 5: note = X at position 5 can be any amino acid except C
  SITE 14: note = X at position 14 can be any amino acid except C
  VARIANT 1..10: note = any one or more of amino acids at any of positions 1-10 may be deleted
EPKSXDTPPPCPRXP

SEQ ID NO: 31 - protein, 5 aa, synthetic construct
  SITE 4: note = X at position 4 can be any amino acid except C
CPRXP

SEQ ID NO: 32 - protein, 15 aa, synthetic construct
  SITE 11: note = X at position 11 can be any amino acid except C
  SITE 14: note = X at position 14 can be any amino acid except C
  VARIANT 1..4: note = any one or more of amino acids at any of positions 1-4 may be deleted
EPKSCDTPPPXPRXP

SEQ ID NO: 33 - protein, 11 aa, synthetic construct
  SITE 7: note = X at position 7 can be any amino acid except C
  SITE 10: note = X at position 10 can be any amino acid except C
CDTPPPXPRXP

SEQ ID NO: 34 - protein, 15 aa, synthetic construct
  SITE 5: note = X at position 5 can be any amino acid except C
  SITE 11: note = X at position 11 can be any amino acid except C
  SITE 7: note = X at position 7 can be any amino acid except C or T
  VARIANT 1..11: note = any one or more of amino acids at any of positions 1-11 may be deleted
EPKSXDXPPPXPRCP

SEQ ID NO: 35 - protein, 15 aa, synthetic construct
  SITE 5: note = X at position 5 can be any amino acid except C
  SITE 14: note = X at position 14 can be any amino acid except C
  SITE 7: note = X at position 7 can be any amino acid except C or T
  VARIANT 1..10: note = any one or more of amino acids at any of positions 1-10 may be deleted
EPKSXDXPPPCPRXP

SEQ ID NO: 36 - protein, 15 aa, synthetic construct
  SITE 11: note = X at position 11 can be any amino acid except C
  SITE 14: note = X at position 14 can be any amino acid except C
  SITE 7: note = X at position 7 can be any amino acid except C or T
  VARIANT 1..4: note = any one or more of amino acids at any of positions 1-4 may be deleted
EPKSCDXPPPXPRXP

SEQ ID NO: 37 - protein, 11 aa, synthetic construct
  SITE 7: note = X at position 7 can be any amino acid except C
  SITE 10: note = X at position 10 can be any amino acid except C
  SITE 3: note = X at position 3 can be any amino acid except C or T
CDXPPPXPRXP

SEQ ID NO: 38 - protein, 15 aa, synthetic construct
  SITE 5: note = X at position 5 can be any amino acid except C
  SITE 11: note = X at position 11 can be any amino acid except C
  SITE 4: note = X at position 4 can be any amino acid except C, T or S
  VARIANT 1..11: note = any one or more of amino acids at any of positions 1-11 may be deleted
EPKXXDTPPPXPRCP

SEQ ID NO: 39 - protein, 15 aa, synthetic construct
  SITE 5: note = X at position 5 can be any amino acid except C
  SITE 14: note = X at position 14 can be any amino acid except C
  SITE 4: note = X at position 4 can be any amino acid except C, T or S
  VARIANT 1..10: note = any one or more of amino acids at any of positions 1-10 may be deleted
EPKXXDTPPPCPRXP

SEQ ID NO: 40 - protein, 15 aa, synthetic construct
  SITE 11: note = X at position 11 can be any amino acid except C
  SITE 14: note = X at position 14 can be any amino acid except C
  SITE 4: note = X at position 4 can be any amino acid except C, T or S
  VARIANT 1..4: note = any one or more of amino acids at any of positions 1-4 may be deleted
EPKXCDTPPPXPRXP

SEQ ID NO: 41 - protein, 15 aa, synthetic construct
  SITE 5: note = X at position 5 can be any amino acid except C
  SITE 11: note = X at position 11 can be any amino acid except C
  SITE 4: note = X at position 4 can be any amino acid except C, T or S
  SITE 7: note = X at position 7 can be any amino acid except C or T
  VARIANT 1..11: note = any one or more of amino acids at any of positions 1-11 may be deleted
EPKXXDXPPPXPRCP

SEQ ID NO: 42 - protein, 15 aa, synthetic construct
  SITE 5: note = X at position 5 can be any amino acid except C
  SITE 14: note = X at position 14 can be any amino acid except C
  SITE 4: note = X at position 4 can be any amino acid except C, T or S
  SITE 7: note = X at position 7 can be any amino acid except C or T
  VARIANT 1..10: note = any one or more of amino acids at any of positions 1-10 may be deleted
EPKXXDXPPPCPRXP

SEQ ID NO: 43 - protein, 15 aa, synthetic construct
  SITE 11: note = X at position 11 can be any amino acid except C
  SITE 14: note = X at position 14 can be any amino acid except C
  SITE 4: note = X at position 4 can be any amino acid except C, T or S
  SITE 7: note = X at position 7 can be any amino acid except C or T
  VARIANT 1..4: note = any one or more of amino acids at any of positions 1-4 may be deleted
EPKXCDXPPPXPRXP

SEQ ID NO: 44 - protein, 11 aa, synthetic construct
  SITE 7: note = X at position 7 can be any amino acid except C
  SITE 10: note = X at position 10 can be any amino acid except C
  SITE 3: note = X at position 3 can be any amino acid except C or T
CDXPPPXPRXP

SEQ ID NO: 45 - protein, 15 aa, synthetic construct
  SITE 5: note = X at position 5 can be any amino acid except C
  VARIANT 1..10: note = any one or more of amino acids at any of positions 1-10 may be deleted
EPKSXDTPPPCPRCP

SEQ ID NO: 46 - protein, 5 aa, synthetic construct
CPRCP

SEQ ID NO: 47 - protein, 15 aa, synthetic construct
  SITE 11: note = X at position 11 can be any amino acid except C
  VARIANT 1..4: note = any one or more of amino acids at any of positions 1-4 may be deleted
EPKSCDTPPPXPRCP

SEQ ID NO: 48 - protein, 11 aa, synthetic construct
  SITE 7: note = X at position 7 can be any amino acid except C
CDTPPPXPRCP

SEQ ID NO: 49 - protein, 15 aa, synthetic construct
  SITE 14: note = X at position 14 can be any amino acid except C
  VARIANT 1..4: note = any one or more of amino acids at any of positions 1-4 may be deleted
EPKSCDTPPPCPRXP

SEQ ID NO: 50 - protein, 11 aa, synthetic construct
  SITE 10: note = X at position 10 can be any amino acid except C
CDTPPPCPRXP

SEQ ID NO: 51 - protein, 15 aa, synthetic construct
  SITE 5: note = X at position 5 can be any amino acid except C
  SITE 7: note = X at position 7 can be any amino acid except C or T
  VARIANT 1..10: note = any one or more of amino acids at any of positions 1-10 may be deleted
EPKSXDXPPPCPRCP

SEQ ID NO: 52 - protein, 15 aa, synthetic construct
  SITE 11: note = X at position 11 can be any amino acid except C
  SITE 7: note = X at position 7 can be any amino acid except C or T
  VARIANT 1..4: note = any one or more of amino acids at any of positions 1-4 may be deleted
EPKSCDXPPPXPRCP

SEQ ID NO: 53 - protein, 11 aa, synthetic construct
  SITE 3: note = X at position 3 can be any amino acid except C or T
  SITE 7: note = X at position 7 can be any amino acid except C
CDXPPPXPRCP

SEQ ID NO: 54 - protein, 15 aa, synthetic construct
  SITE 14: note = X at position 14 can be any amino acid except C
  SITE 7: note = X at position 7 can be any amino acid except C or T
  VARIANT 1..4: note = any one or more of amino acids at any of positions 1-4 may be deleted
EPKSCDXPPPCPRXP

SEQ ID NO: 55 - protein, 11 aa, synthetic construct
  SITE 3: note = X at position 3 can be any amino acid except C or T
  SITE 10: note = X at position 10 can be any amino acid except C
CDXPPPCPRXP

SEQ ID NO: 56 - protein, 15 aa, synthetic construct
  SITE 5: note = X at position 5 can be any amino acid except C
  SITE 4: note = X at position 4 can be any amino acid except C, T or S
  VARIANT 1..10: note = any one or more of amino acids at any of positions 1-10 may be deleted
EPKXXDTPPPCPRCP

SEQ ID NO: 57 - protein, 15 aa, synthetic construct
  SITE 11: note = X at position 11 can be any amino acid except C
  SITE 4: note = X at position 4 can be any amino acid except C, T or S
  VARIANT 1..4: note = any one or more of amino acids at any of positions 1-4 may be deleted
EPKXCDTPPPXPRCP

SEQ ID NO: 58 - protein, 15 aa, synthetic construct
  SITE 14: note = X at position 14 can be any amino acid except C
  SITE 4: note = X at position 4 can be any amino acid except C, T or S
  VARIANT 1..4: note = any one or more of amino acids at any of positions 1-4 may be deleted
EPKXCDTPPPCPRXP

SEQ ID NO: 59 - protein, 15 aa, synthetic construct
  SITE 5: note = X at position 5 can be any amino acid except C
  SITE 4: note = X at position 4 can be any amino acid except C, T or S
  SITE 7: note = X at position 7 can be any amino acid except C or T
  VARIANT 1..10: note = any one or more of amino acids at any of positions 1-10 may be deleted
EPKXXDXPPPCPRCP

SEQ ID NO: 60 - protein, 15 aa, synthetic construct
  SITE 11: note = X at position 11 can be any amino acid except C
  SITE 4: note = X at position 4 can be any amino acid except C, T or S
  SITE 7: note = X at position 7 can be any amino acid except C or T
  VARIANT 1..4: note = any one or more of amino acids at any of positions 1-4 may be deleted
EPKXCDXPPPXPRCP

SEQ ID NO: 61 - protein, 15 aa, synthetic construct
  SITE 14: note = X at position 14 can be any amino acid except C
  SITE 4: note = X at position 4 can be any amino acid except C, T or S
  SITE 7: note = X at position 7 can be any amino acid except C or T
  VARIANT 1..4: note = any one or more of amino acids at any of positions 1-4 may be deleted
EPKXCDXPPPCPRXP

SEQ ID NO: 62 - protein, 15 aa, synthetic construct
  VARIANT 1..4: note = any one or more of amino acids at any of positions 1-4 may be deleted
EPKSCDTPPPCPRCP

SEQ ID NO: 63 - protein, 11 aa, synthetic construct
CDTPPPCPRCP

SEQ ID NO: 64 - protein, 15 aa, synthetic construct
  SITE 7: note = X at position 7 can be any amino acid except C or T
  VARIANT 1..4: note = any one or more of amino acids at any of positions 1-4 may be deleted
EPKSCDXPPPCPRCP

SEQ ID NO: 65 - protein, 11 aa, synthetic construct
  SITE 3: note = X at position 3 can be any amino acid except C or T
CDXPPPCPRCP

SEQ ID NO: 66 - protein, 15 aa, synthetic construct
  SITE 4: note = X at position 4 can be any amino acid except C, T or S
  VARIANT 1..4: note = any one or more of amino acids at any of positions 1-4 may be deleted
EPKXCDTPPPCPRCP

SEQ ID NO: 67 - protein, 15 aa, synthetic construct
  SITE 4: note = X at position 4 can be any amino acid except C, T or S
  SITE 7: note = X at position 7 can be any amino acid except C or T
  VARIANT 1..4: note = any one or more of amino acids at any of positions 1-4 may be deleted
EPKXCDXPPPCPRCP

SEQ ID NO: 68 - protein, 19 aa, synthetic construct
  VARIANT 1..2: note = any one or more of amino acids at any of positions 1-2 may be deleted
PRCPEPKSCDTPPPCPRCP

SEQ ID NO: 69 - protein, 17 aa, synthetic construct
CPEPKSCDTPPPCPRCP

SEQ ID NO: 70 - protein, 19 aa, synthetic construct
  SITE 11: note = X at position 11 can be any amino acid except C or T
  VARIANT 1..2: note = any one or more of amino acids at any of positions 1-2 may be deleted
PRCPEPKSCDXPPPCPRCP

SEQ ID NO: 71 - protein, 17 aa, synthetic construct
  SITE 9: note = X at position 9 can be any amino acid except C or T
CPEPKSCDXPPPCPRCP

SEQ ID NO: 72 - protein, 19 aa, synthetic construct
  SITE 8: note = X at position 8 can be any amino acid except C, T or S
  VARIANT 1..2: note = any one or more of amino acids at any of positions 1-2 may be deleted
PRCPEPKXCDTPPPCPRCP

SEQ ID NO: 73 - protein, 17 aa, synthetic construct
  SITE 6: note = X at position 6 can be any amino acid except C, T or S
CPEPKXCDTPPPCPRCP

SEQ ID NO: 74 - protein, 19 aa, synthetic construct
  SITE 8: note = X at position 8 can be any amino acid except C, T or S
  SITE 11: note = X at position 11 can be any amino acid except C or T
  VARIANT 1..2: note = any one or more of amino acids at any of positions 1-2 may be deleted
PRCPEPKXCDXPPPCPRCP

SEQ ID NO: 75 - protein, 17 aa, synthetic construct
  SITE 6: note = X at position 6 can be any amino acid except C, T or S
  SITE 9: note = X at position 9 can be any amino acid except C or T
CPEPKXCDXPPPCPRCP

SEQ ID NO: 76 - protein, 25 aa, synthetic construct
  VARIANT 1..5: note = any one or more of amino acids at any of positions 1-5 may be deleted
DTPPPCPRCPEPKSCDTPPPCPRCP

SEQ ID NO: 77 - protein, 20 aa, synthetic construct
CPRCPEPKSCDTPPPCPRCP

SEQ ID NO: 78 - protein, 25 aa, synthetic construct
  SITE 17: note = X at position 17 can be any amino acid except C or T
  VARIANT 1..5: note = any one or more of amino acids at any of positions 1-5 may be deleted
DTPPPCPRCPEPKSCDXPPPCPRCP

SEQ ID NO: 79 - protein, 20 aa, synthetic construct
  SITE 12: note = X at position 12 can be any amino acid except C or T
CPRCPEPKSCDXPPPCPRCP

SEQ ID NO: 80 - protein, 25 aa, synthetic construct
  SITE 2: note = X at position 2 can be any amino acid except C or T
  VARIANT 1..5: note = any one or more of amino acids at any of positions 1-5 may be deleted
DXPPPCPRCPEPKSCDTPPPCPRCP

SEQ ID NO: 81 - protein, 25 aa, synthetic construct
  SITE 2: note = X at position 2 can be any amino acid except C or T
  SITE 17: note = X at position 17 can be any amino acid except C or T
  VARIANT 1..5: note = any one or more of amino acids at any of positions 1-5 may be deleted
DXPPPCPRCPEPKSCDXPPPCPRCP

SEQ ID NO: 82 - protein, 25 aa, synthetic construct
  SITE 14: note = the X at position 14 can be any amino acid except C, T or S
  VARIANT 1..5: note = any one or more of amino acids at any of positions 1-5 may be deleted
DTPPPCPRCPEPKXCDTPPPCPRCP

SEQ ID NO: 83 - protein, 20 aa, synthetic construct
  SITE 9: note = X at position 9 can be any amino acid except C, T or S
CPRCPEPKXCDTPPPCPRCP

SEQ ID NO: 84 - protein, 25 aa, synthetic construct
  SITE 2: note = X at position 2 can be any amino acid except C or T
  SITE 14: note = X at position 14 can be any amino acid except C, T or S
  SITE 17: note = X at position 17 can be any amino acid except C or T
  VARIANT 1..5: note = any one or more of amino acids at any of positions 1-5 may be deleted
DXPPPCPRCPEPKXCDXPPPCPRCP

SEQ ID NO: 85 - protein, 20 aa, synthetic construct
  SITE 9: note = X at position 9 can be any amino acid except C, T or S
  SITE 12: note = X at position 12 can be any amino acid except C or T
CPRCPEPKXCDXPPPCPRCP

SEQ ID NO: 86 - protein, 25 aa, synthetic construct
  SITE 2: note = X at position 2 can be any amino acid except C or T
  SITE 14: note = X at position 14 can be any amino acid except C, T or S
  VARIANT 1..5: note = any one or more of amino acids at any of positions 1-5 may be deleted
DXPPPCPRCPEPKXCDTPPPCPRCP

SEQ ID NO: 87 - protein, 25 aa, synthetic construct
  SITE 14: note = X at position 14 can be any amino acid except C, T or S
  SITE 17: note = X at position 17 can be any amino acid except C or T
  VARIANT 1..5: note = any one or more of amino acids at any of positions 1-5 may be deleted
DTPPPCPRCPEPKXCDXPPPCPRCP

SEQ ID NO: 88 - protein, 30 aa, synthetic construct
  VARIANT 1..4: note = any one or more of amino acids at any of positions 1-4 may be deleted
EPKSCDTPPPCPRCPEPKSCDTPPPCPRCP

SEQ ID NO: 89 - protein, 26 aa, synthetic construct
CDTPPPCPRCPEPKSCDTPPPCPRCP

SEQ ID NO: 90 - protein, 30 aa, synthetic construct
  SITE 7: note = X at position 7 can be any amino acid except C or T
  VARIANT 1..4: note = any one or more of amino acids at any of positions 1-4 may be deleted
EPKSCDXPPPCPRCPEPKSCDTPPPCPRCP

SEQ ID NO: 91 - protein, 26 aa, synthetic construct
  SITE 3: note = X at position 3 can be any amino acid except C or T
CDXPPPCPRCPEPKSCDTPPPCPRCP

SEQ ID NO: 92 - protein, 30 aa, synthetic construct
  SITE 22: note = X at position 22 can be any amino acid except C or T
  VARIANT 1..4: note = any one or more of amino acids at any of positions 1-4 may be deleted
EPKSCDTPPPCPRCPEPKSCDXPPPCPRCP

SEQ ID NO: 93 - protein, 26 aa, synthetic construct
  SITE 18: note = X at position 18 can be any amino acid except C or T
CDTPPPCPRCPEPKSCDXPPPCPRCP

SEQ ID NO: 94 - protein, 30 aa, synthetic construct
  SITE 7: note = X at position 7 can be any amino acid except C or T
  SITE 22: note = X at position 22 can be any amino acid except C or T
  VARIANT 1..4: note = any one or more of amino acids at any of positions 1-4 may be deleted
EPKSCDXPPPCPRCPEPKSCDXPPPCPRCP

SEQ ID NO: 95 - protein, 26 aa, synthetic construct
  SITE 3: note = X at position 3 can be any amino acid except C or T
  SITE 18: note = X at position 18 can be any amino acid except C or T
CDXPPPCPRCPEPKSCDXPPPCPRCP

SEQ ID NO: 96 - protein, 30 aa, synthetic construct
  SITE 4: note = X at position 4 can be any amino acid except C, T or S
  VARIANT 1..4: note = any one or more of amino acids at any of positions 1-4 may be deleted
EPKXCDTPPPCPRCPEPKSCDTPPPCPRCP

SEQ ID NO: 97 - protein, 30 aa, synthetic construct
  SITE 19: note = X at position 19 can be any amino acid except C, T or S
  VARIANT 1..4: note = any one or more of amino acids at any of positions 1-4 may be deleted
EPKSCDTPPPCPRCPEPKXCDTPPPCPRCP

SEQ ID NO: 98 - protein, 26 aa, synthetic construct
  SITE 15: note = X at position 15 can be any amino acid except C, T or S
CDTPPPCPRCPEPKXCDTPPPCPRCP

SEQ ID NO: 99 - protein, 30 aa, synthetic construct
  SITE 4: note = X at position 4 can be any amino acid except C, T or S
  SITE 19: note = X at position 19 can be any amino acid except C, T or S
  VARIANT 1..4: note = any one or more of amino acids at any of positions 1-4 may be deleted
EPKXCDTPPPCPRCPEPKXCDTPPPCPRCP

SEQ ID NO: 100 - protein, 30 aa, synthetic construct
  SITE 4: note = X at position 4 can be any amino acid except C, T or S
  SITE 7: note = X at position 7 can be any amino acid except C or T
  SITE 19: note = X at position 19 can be any amino acid except C, T or S
  SITE 22: note = X at position 22 can be any amino acid except C or T
  VARIANT 1..4: note = any one or more of amino acids at any of positions 1-4 may be deleted
EPKXCDXPPPCPRCPEPKXCDXPPPCPRCP

SEQ ID NO: 101 - protein, 26 aa, synthetic construct
  SITE 3: note = X at position 3 can be any amino acid except C or T
  SITE 15: note = X at position 15 can be any amino acid except C, T or S
  SITE 18: note = X at position 18 can be any amino acid except C or T
CDXPPPCPRCPEPKXCDXPPPCPRCP

SEQ ID NO: 102 - protein, 30 aa, synthetic construct
  SITE 4: note = X at position 4 can be any amino acid except C, T or S
  SITE 7: note = X at position 7 can be any amino acid except C or T
  SITE 19: note = X at position 19 can be any amino acid except C, T or S
  VARIANT 1..4: note = any one or more of amino acids at any of positions 1-4 may be deleted
EPKXCDXPPPCPRCPEPKXCDTPPPCPRCP

SEQ ID NO: 103 - protein, 26 aa, synthetic construct
  SITE 3: note = X at position 3 can be any amino acid except C or T
  SITE 15: note = X at position 15 can be any amino acid except C, T or S
CDXPPPCPRCPEPKXCDTPPPCPRCP

SEQ ID NO: 104 - protein, 30 aa, synthetic construct
  SITE 4: note = X at position 4 can be any amino acid except C, T or S
  SITE 7: note = X at position 7 can be any amino acid except C or T
  SITE 22: note = X at position 22 can be any amino acid except C or T
  VARIANT 1..4: note = any one or more of amino acids at any of positions 1-4 may be deleted
EPKXCDXPPPCPRCPEPKSCDXPPPCPRCP

SEQ ID NO: 105 - protein, 30 aa, synthetic construct
  SITE 4: note = X at position 4 can be any amino acid except C, T or S
  SITE 19: note = X at position 19 can be any amino acid except C, T or S
  SITE 22: note = X at position 22 can be any amino acid except C or T
  VARIANT 1..4: note = any one or more of amino acids at any of positions 1-4 may be deleted
EPKXCDTPPPCPRCPEPKXCDXPPPCPRCP

SEQ ID NO: 106 - protein, 26 aa, synthetic construct
  SITE 15: note = X at position 15 can be any amino acid except C, T or S
  SITE 18: note = X at position 18 can be any amino acid except C or T
CDTPPPCPRCPEPKXCDXPPPCPRCP

SEQ ID NO: 107 - protein, 30 aa, synthetic construct
  SITE 7: note = X at position 7 can be any amino acid except C or T
  SITE 19: note = X at position 19 can be any amino acid except C, T or S
  SITE 22: note = X at position 22 can be any amino acid except C or T
  VARIANT 1..4: note = any one or more of amino acids at any of positions 1-4 may be deleted
EPKSCDXPPPCPRCPEPKXCDXPPPCPRCP

SEQ ID NO: 108 - protein, 30 aa, synthetic construct
  SITE 4: note = X at position 4 can be any amino acid except C, T or S
  SITE 7: note = X at position 7 can be any amino acid except C or T
  VARIANT 1..4: note = any one or more of amino acids at any of positions 1-4 may be deleted
EPKXCDXPPPCPRCPEPKSCDTPPPCPRCP

SEQ ID NO: 109 - protein, 30 aa, synthetic construct
  SITE 4: note = X at position 4 can be any amino acid except C, T or S
  SITE 22: note = X at position 22 can be any amino acid except C or T
  VARIANT 1..4: note = any one or more of amino acids at any of positions 1-4 may be deleted
EPKXCDTPPPCPRCPEPKSCDXPPPCPRCP

SEQ ID NO: 110 - protein, 30 aa, synthetic construct
  SITE 7: note = X at position 7 can be any amino acid except C or T
  SITE 19: note = X at position 19 can be any amino acid except C, T or S
  VARIANT 1..4: note = any one or more of amino acids at any of positions 1-4 may be deleted
EPKSCDXPPPCPRCPEPKXCDTPPPCPRCP

SEQ ID NO: 111 - protein, 30 aa, synthetic construct
  SITE 19: note = X at position 19 can be any amino acid except C, T or S
  SITE 22: note = X at position 22 can be any amino acid except C or T
EPKSCDTPPPCPRCPEPKXCDXPPPCPRCP

SEQ ID NO: 112 - protein, 19 aa, synthetic construct
PRCPEPKACDAPPPCPRCP

SEQ ID NO: 113 - protein, 10 aa, synthetic construct
  SITE 2: note = X at position 2 can be any amino acid except C or T
DXPPPCPRCP

SEQ ID NO: 114 - protein, 12 aa, synthetic construct
  SITE 8: note = X at position 8 can be any amino acid except C
ESKYGPPXPSCP

SEQ ID NO: 115 - protein, 12 aa, synthetic construct
  SITE 11: note = X at position 11 can be any amino acid except C
ESKYGPPCPSXP

SEQ ID NO: 116 - protein, 12 aa, synthetic construct
  SITE 8: note = X at position 8 can be any amino acid except C
  SITE 10: note = X at position 10 can be any amino acid except C
ESKYGPPXPXCP

SEQ ID NO: 117 - protein, 12 aa, synthetic construct
  SITE 11: note = X at position 11 can be any amino acid except C
  SITE 10: note = X at position 10 can be any amino acid except C
ESKYGPPCPXXP

SEQ ID NO: 118 - protein, 12 aa, synthetic construct
  SITE 10: note = X at position 10 can be any amino acid except C
ESKYGPPCPXCP